European Patent Application EP 4 512 896 A1, published February 26, 2025. Title: A Method for detecting molecular interactions in a biological sample and a kit thereof. Applicant: 大阪大学. The sequence listing filed with the application follows.

SEQUENCE LISTING (88 sequences)

SEQ ID NO: 1 - skipped

SEQ ID NO: 2 - DNA, 66 bp, synthetic construct
  misc_feature 17..23: note = n stands for any base
  misc_feature 27..29: note = n stands for any base
  misc_feature 33..36: note = n stands for any base
  source 1..66: mol_type = other DNA
gacgctcttccgatctnnnnnnnwwsnnnwwwnnnnsaccttttggcgtaagtttaggacacctca

SEQ ID NO: 3 - DNA, 66 bp, synthetic construct
  misc_feature 17..23: note = n stands for any base
  misc_feature 27..29: note = n stands for any base
  misc_feature 33..36: note = n stands for any base
  source 1..66: mol_type = other DNA
gacgctcttccgatctnnnnnnnwwsnnnwwwnnnnsacgctaccgcgtaagtttaggacacctca

SEQ ID NO: 4 - DNA, 66 bp, synthetic construct
  misc_feature 17..23: note = n stands for any base
  misc_feature 27..29: note = n stands for any base
  misc_feature 33..36: note = n stands for any base
  source 1..66: mol_type = other DNA
gacgctcttccgatctnnnnnnnwwsnnnwwwnnnnsacgctcatgcgtaagtttaggacacctca

SEQ ID NO: 5 - DNA, 66 bp, synthetic construct
  misc_feature 17..23: note = n stands for any base
  misc_feature 27..29: note = n stands for any base
  misc_feature 33..36: note = n stands for any base
  source 1..66: mol_type = other DNA
tgtgctcttccgatctnnnnnnnwwsnnnwwwnnnnsaccgtgatgcgatatgttgagaccactcc

SEQ ID NO: 6 - skipped

SEQ ID NO: 7 - DNA, 52 bp, synthetic construct
  misc_feature 19..23: note = n stands for any base
  misc_feature 26..30: note = n stands for any base
  source 1..52: mol_type = other DNA
  misc_feature 1..52: note = Primer
tattcccatggcgcgccannnnnatnnnnnttgaggtgtcctaaacttacgc

SEQ ID NO: 8 - DNA, 52 bp, synthetic construct
  misc_feature 19..23: note = n stands for any base
  misc_feature 26..30: note = n stands for any base
  source 1..52: mol_type = other DNA
  misc_feature 1..52: note = Primer
ggcgcgccatgggaataannnnnatnnnnntggagtggtctcaacatatcgc

SEQ ID NO: 9 - DNA, 25 bp, synthetic construct
  source 1..25: mol_type = other DNA
  misc_feature 1..25: note = Primer
tccctacacgacgctcttccgatct

SEQ ID NO: 10 - DNA, 25 bp, synthetic construct
  source 1..25: mol_type = other DNA
  misc_feature 1..25: note = Primer
gttcagacgtgtgctcttccgatct

SEQ ID NO: 11 - DNA, 58 bp, synthetic construct
  source 1..58: mol_type = other DNA
  misc_feature 1..58: note = Primer
aatgatacggcgaccaccgagatctacactctttccctacacgacgctcttccgatct

SEQ ID NO: 12 - DNA, 64 bp, synthetic construct
  misc_feature 25..30: note = n stands for any base
  source 1..64: mol_type = other DNA
  misc_feature 1..64: note = Primer
caagcagaagacggcatacgagatnnnnnngtgactggagttcagacgtgtgctcttccgatct

SEQ ID NO: 13 - DNA, 19 bp, synthetic construct
  source 1..19: mol_type = other DNA
  misc_feature 1..19: note = Primer
tggcgcgccatgggaataa

SEQ ID NO: 14 - DNA, 19 bp, synthetic construct
  source 1..19: mol_type = other DNA
  misc_feature 1..19: note = Primer
ttattcccatggcgcgcca

SEQ ID NO: 15 - DNA, 66 bp, synthetic construct
  misc_feature 17..23: note = n stands for any base
  misc_feature 27..29: note = n stands for any base
  misc_feature 33..36: note = n stands for any base
  source 1..66: mol_type = other DNA
gacgctcttccgatctnnnnnnnwwsnnnwwwnnnnsaccgtgatgcgtaagtttaggacacctca

SEQ ID NO: 16 - DNA, 66 bp, synthetic construct
  misc_feature 17..23: note = n stands for any base
  misc_feature 27..29: note = n stands for any base
  misc_feature 33..36: note = n stands for any base
  source 1..66: mol_type = other DNA
gacgctcttccgatctnnnnnnnwwsnnnwwwnnnnsacacatcggcgtaagtttaggacacctca

SEQ ID NO: 17 - DNA, 66 bp, synthetic construct
  misc_feature 17..23: note = n stands for any base
  misc_feature 27..29: note = n stands for any base
  misc_feature 33..36: note = n stands for any base
  source 1..66: mol_type = other DNA
gacgctcttccgatctnnnnnnnwwsnnnwwwnnnnsacgcctaagcgtaagtttaggacacctca

SEQ ID NO: 18 - DNA, 66 bp, synthetic construct
  misc_feature 17..23: note = n stands for any base
  misc_feature 27..29: note = n stands for any base
  misc_feature 33..36: note = n stands for any base
  source 1..66: mol_type = other DNA
gacgctcttccgatctnnnnnnnwwsnnnwwwnnnnsactggtcagcgtaagtttaggacacctca

SEQ ID NO: 19 - DNA, 66 bp, synthetic construct
  misc_feature 17..23: note = n stands for any base
  misc_feature 27..29: note = n stands for any base
  misc_feature 33..36: note = n stands for any base
  source 1..66: mol_type = other DNA
gacgctcttccgatctnnnnnnnwwsnnnwwwnnnnsactcaagtgcgtaagtttaggacacctca

SEQ ID NO: 20 - DNA, 66 bp, synthetic construct
  misc_feature 17..23: note = n stands for any base
  misc_feature 27..29: note = n stands for any base
  misc_feature 33..36: note = n stands for any base
  source 1..66: mol_type = other DNA
tgtgctcttccgatctnnnnnnnwwsnnnwwwnnnnsacctctacgcgatatgttgagaccactcc

SEQ ID NO: 21 - DNA, 66 bp, synthetic construct
  misc_feature 17..23: note = n stands for any base
  misc_feature 27..29: note = n stands for any base
  misc_feature 33..36: note = n stands for any base
  source 1..66: mol_type = other DNA
tgtgctcttccgatctnnnnnnnwwsnnnwwwnnnnsacgctaccgcgatatgttgagaccactcc

SEQ ID NO: 22 - DNA, 66 bp, synthetic construct
  misc_feature 17..23: note = n stands for any base
  misc_feature 27..29: note = n stands for any base
  misc_feature 33..36: note = n stands for any base
  source 1..66: mol_type = other DNA
tgtgctcttccgatctnnnnnnnwwsnnnwwwnnnnsacgctcatgcgatatgttgagaccactcc

SEQ ID NO: 23 - DNA, 66 bp, synthetic construct
  misc_feature 17..23: note = n stands for any base
  misc_feature 27..29: note = n stands for any base
  misc_feature 33..36: note = n stands for any base
  source 1..66: mol_type = other DNA
tgtgctcttccgatctnnnnnnnwwsnnnwwwnnnnsaccttttggcgatatgttgagaccactcc

SEQ ID NO: 24 - DNA, 66 bp, synthetic construct
  misc_feature 17..23: note = n stands for any base
  misc_feature 27..29: note = n stands for any base
  misc_feature 33..36: note = n stands for any base
  source 1..66: mol_type = other DNA
tgtgctcttccgatctnnnnnnnwwsnnnwwwnnnnsacatcgtggcgatatgttgagaccactcc

SEQ ID NO: 25 - DNA, 66 bp, synthetic construct
  misc_feature 17..23: note = n stands for any base
  misc_feature 27..29: note = n stands for any base
  misc_feature 33..36: note = n stands for any base
  source 1..66: mol_type = other DNA
gacgctcttccgatctnnnnnnnwwsnnnwwwnnnnsaccactgtgcgtaagtttaggacacctca

SEQ ID NO: 26 - DNA, 66 bp, synthetic construct
  misc_feature 17..23: note = n stands for any base
  misc_feature 27..29: note = n stands for any base
  misc_feature 33..36: note = n stands for any base
  source 1..66: mol_type = other DNA
tgtgctcttccgatctnnnnnnnwwsnnnwwwnnnnsactagttggcgatatgttgagaccactcc

SEQ ID NO: 27 - DNA, 66 bp, synthetic construct; identical to SEQ ID NO: 19
  source 1..66: mol_type = other DNA
  misc_feature 17..23: note = n stands for any base
  misc_feature 27..29: note = n stands for any base
  misc_feature 33..36: note = n stands for any base

SEQ ID NO: 28 - DNA, 66 bp, synthetic construct
  source 1..66: mol_type = other DNA
  misc_feature 17..23: note = n stands for any base
  misc_feature 27..29: note = n stands for any base
  misc_feature 33..36: note = n stands for any base
gacgctcttccgatctnnnnnnnwwsnnnwwwnnnnsacctgatcgcgtaagtttaggacacctca

SEQ ID NO: 29 - DNA, 66 bp, synthetic construct
  source 1..66: mol_type = other DNA
  misc_feature 17..23: note = n stands for any base
  misc_feature 27..29: note = n stands for any base
  misc_feature 33..36: note = n stands for any base
gacgctcttccgatctnnnnnnnwwsnnnwwwnnnnsacaagctagcgtaagtttaggacacctca

SEQ ID NO: 30 - DNA, 66 bp, synthetic construct
  source 1..66: mol_type = other DNA
  misc_feature 17..23: note = n stands for any base
  misc_feature 33..36: note = n stands for any base
  misc_feature 27..29: note = n stands for any base
gacgctcttccgatctnnnnnnnwwsnnnwwwnnnnsacgatctggcgtaagtttaggacacctca

SEQ ID NO: 31 - DNA, 66 bp, synthetic construct
  source 1..66: mol_type = other DNA
  misc_feature 17..23: note = n stands for any base
  misc_feature 27..29: note = n stands for any base
  misc_feature 33..36: note = n stands for any base
gacgctcttccgatctnnnnnnnwwsnnnwwwnnnnsacgtagccgcgtaagtttaggacacctca

SEQ ID NO: 32 - DNA, 66 bp, synthetic construct
  source 1..66: mol_type = other DNA
  misc_feature 17..23: note = n stands for any base
  misc_feature 27..29: note = n stands for any base
  misc_feature 33..36: note = n stands for any base
gacgctcttccgatctnnnnnnnwwsnnnwwwnnnnsactacaaggcgtaagtttaggacacctca

SEQ ID NO: 33 - DNA, 68 bp, synthetic construct
  source 1..68: mol_type = other DNA
  misc_feature 17..23: note = n stands for any base
  misc_feature 27..29: note = n stands for any base
  misc_feature 33..36: note = n stands for any base
gacgctcttccgatctnnnnnnnwwsnnnwwwnnnnsactgttgactgcgtaagtttaggacacctca

SEQ ID NO: 34 - DNA, 68 bp, synthetic construct
  source 1..68: mol_type = other DNA
  misc_feature 17..23: note = n stands for any base
  misc_feature 27..29: note = n stands for any base
  misc_feature 33..36: note = n stands for any base
gacgctcttccgatctnnnnnnnwwsnnnwwwnnnnsacacggaactgcgtaagtttaggacacctca

SEQ ID NO: 35 - DNA, 68 bp, synthetic construct
  source 1..68: mol_type = other DNA
  misc_feature 17..23: note = n stands for any base
  misc_feature 27..29: note = n stands for any base
  misc_feature 33..36: note = n stands for any base
gacgctcttccgatctnnnnnnnwwsnnnwwwnnnnsactctgacatgcgtaagtttaggacacctca

SEQ ID NO: 36 - DNA, 66 bp, synthetic construct
  source 1..66: mol_type = other DNA
  misc_feature 17..23: note = n stands for any base
  misc_feature 27..29: note = n stands for any base
  misc_feature 33..36: note = n stands for any base
gacgctcttccgatctnnnnnnnwwsnnnwwwnnnnsacggacgggcgtaagtttaggacacctca

SEQ ID NO: 37 - DNA, 68 bp, synthetic construct
  source 1..68: mol_type = other DNA
  misc_feature 17..23: note = n stands for any base
  misc_feature 27..29: note = n stands for any base
  misc_feature 33..36: note = n stands for any base
gacgctcttccgatctnnnnnnnwwsnnnwwwnnnnsacgtgcggacgcgtaagtttaggacacctca

SEQ ID NO: 38 - DNA, 66 bp, synthetic construct
  source 1..66: mol_type = other DNA
  misc_feature 17..23: note = n stands for any base
  misc_feature 27..29: note = n stands for any base
  misc_feature 33..36: note = n stands for any base
tgtgctcttccgatctnnnnnnnwwsnnnwwwnnnnsaccgcctggcgatatgttgagaccactcc

SEQ ID NO: 39 - DNA, 66 bp, synthetic construct
  source 1..66: mol_type = other DNA
  misc_feature 17..23: note = n stands for any base
  misc_feature 27..29: note = n stands for any base
  misc_feature 33..36: note = n stands for any base
tgtgctcttccgatctnnnnnnnwwsnnnwwwnnnnsacgtcgtcgcgatatgttgagaccactcc

SEQ ID NO: 40 - DNA, 66 bp, synthetic construct
  source 1..66: mol_type = other DNA
  misc_feature 17..23: note = n stands for any base
  misc_feature 27..29: note = n stands for any base
  misc_feature 33..36: note = n stands for any base
tgtgctcttccgatctnnnnnnnwwsnnnwwwnnnnsacaaaatggcgatatgttgagaccactcc

SEQ ID NO: 41 - DNA, 66 bp, synthetic construct
  source 1..66: mol_type = other DNA
  misc_feature 17..23: note = n stands for any base
  misc_feature 27..29: note = n stands for any base
  misc_feature 33..36: note = n stands for any base
tgtgctcttccgatctnnnnnnnwwsnnnwwwnnnnsactgagtggcgatatgttgagaccactcc

SEQ ID NO: 42 - DNA, 66 bp, synthetic construct
  source 1..66: mol_type = other DNA
  misc_feature 17..23: note = n stands for any base
  misc_feature 27..29: note = n stands for any base
  misc_feature 33..36: note = n stands for any base
tgtgctcttccgatctnnnnnnnwwsnnnwwwnnnnsactgttgggcgatatgttgagaccactcc

SEQ ID NO: 43 - DNA, 66 bp, synthetic construct
  source 1..66: mol_type = other DNA
  misc_feature 17..23: note = n stands for any base
  misc_feature 27..29: note = n stands for any base
  misc_feature 33..36: note = n stands for any base
tgtgctcttccgatctnnnnnnnwwsnnnwwwnnnnsaccgattagcgatatgttgagaccactcc

SEQ ID NO: 44 - DNA, 66 bp, synthetic construct
  source 1..66: mol_type = other DNA
  misc_feature 17..23: note = n stands for any base
  misc_feature 27..29: note = n stands for any base
  misc_feature 33..36: note = n stands for any base
tgtgctcttccgatctnnnnnnnwwsnnnwwwnnnnsacccggtggcgatatgttgagaccactcc

SEQ ID NO: 45 - DNA, 66 bp, synthetic construct
  source 1..66: mol_type = other DNA
  misc_feature 17..23: note = n stands for any base
  misc_feature 27..29: note = n stands for any base
  misc_feature 33..36: note = n stands for any base
tgtgctcttccgatctnnnnnnnwwsnnnwwwnnnnsacattccggcgatatgttgagaccactcc

SEQ ID NO: 46 - DNA, 66 bp, synthetic construct
  source 1..66: mol_type = other DNA
  misc_feature 17..23: note = n stands for any base
  misc_feature 27..29: note = n stands for any base
  misc_feature 33..36: note = n stands for any base
tgtgctcttccgatctnnnnnnnwwsnnnwwwnnnnsacagctaggcgatatgttgagaccactcc

SEQ ID NO: 47 - DNA, 66 bp, synthetic construct
  source 1..66: mol_type = other DNA
  misc_feature 17..23: note = n stands for any base
  misc_feature 27..29: note = n stands for any base
  misc_feature 33..36: note = n stands for any base
tgtgctcttccgatctnnnnnnnwwsnnnwwwnnnnsacgtataggcgatatgttgagaccactcc

SEQ ID NO: 48 - DNA, 68 bp, synthetic construct
  source 1..68: mol_type = other DNA
  misc_feature 17..23: note = n stands for any base
  misc_feature 27..29: note = n stands for any base
  misc_feature 33..36: note = n stands for any base
tgtgctcttccgatctnnnnnnnwwsnnnwwwnnnnsactggatcacgcgatatgttgagaccactcc

SEQ ID NO: 49 - DNA, 66 bp, synthetic construct; identical to SEQ ID NO: 15
  source 1..66: mol_type = other DNA
  misc_feature 17..23: note = n stands for any base
  misc_feature 27..29: note = n stands for any base
  misc_feature 33..36: note = n stands for any base

SEQ ID NO: 50 - DNA, 66 bp, synthetic construct; identical to SEQ ID NO: 16
  source 1..66: mol_type = other DNA
  misc_feature 17..23: note = n stands for any base
  misc_feature 27..29: note = n stands for any base
  misc_feature 33..36: note = n stands for any base

SEQ ID NO: 51 - DNA, 66 bp, synthetic construct; identical to SEQ ID NO: 17
  source 1..66: mol_type = other DNA
  misc_feature 17..23: note = n stands for any base
  misc_feature 27..29: note = n stands for any base
  misc_feature 33..36: note = n stands for any base

SEQ ID NO: 52 - DNA, 66 bp, synthetic construct; identical to SEQ ID NO: 18
  source 1..66: mol_type = other DNA
  misc_feature 17..23: note = n stands for any base
  misc_feature 27..29: note = n stands for any base
  misc_feature 33..36: note = n stands for any base

SEQ ID NO: 53 - DNA, 66 bp, synthetic construct; identical to SEQ ID NO: 25
  source 1..66: mol_type = other DNA
  misc_feature 17..23: note = n stands for any base
  misc_feature 27..29: note = n stands for any base
  misc_feature 33..36: note = n stands for any base

SEQ ID NO: 54 - DNA, 66 bp, synthetic construct
  source 1..66: mol_type = other DNA
  misc_feature 17..23: note = n stands for any base
  misc_feature 27..29: note = n stands for any base
  misc_feature 33..36: note = n stands for any base
gacgctcttccgatctnnnnnnnwwsnnnwwwnnnnsacattggcgcgtaagtttaggacacctca

SEQ ID NO: 55 - DNA, 66 bp, synthetic construct; identical to SEQ ID NO: 30
  source 1..66: mol_type = other DNA
  misc_feature 17..23: note = n stands for any base
  misc_feature 27..29: note = n stands for any base
  misc_feature 33..36: note = n stands for any base

SEQ ID NO: 56 - DNA, 66 bp, synthetic construct; identical to SEQ ID NO: 19
  source 1..66: mol_type = other DNA
  misc_feature 17..23: note = n stands for any base
  misc_feature 27..29: note = n stands for any base
  misc_feature 33..36: note = n stands for any base

SEQ ID NO: 57 - DNA, 66 bp, synthetic construct; identical to SEQ ID NO: 28
  source 1..66: mol_type = other DNA
  misc_feature 27..29: note = n stands for any base
  misc_feature 17..23: note = n stands for any base
  misc_feature 33..36: note = n stands for any base

SEQ ID NO: 58 - DNA, 66 bp, synthetic construct; identical to SEQ ID NO: 29
  source 1..66: mol_type = other DNA
  misc_feature 17..23: note = n stands for any base
  misc_feature 27..29: note = n stands for any base
  misc_feature 33..36: note = n stands for any base

SEQ ID NO: 59 - DNA, 66 bp, synthetic construct; identical to SEQ ID NO: 31
  source 1..66: mol_type = other DNA
  misc_feature 17..23: note = n stands for any base
  misc_feature 27..29: note = n stands for any base
  misc_feature 33..36: note = n stands for any base

SEQ ID NO: 60 - DNA, 66 bp, synthetic construct; identical to SEQ ID NO: 32
  source 1..66: mol_type = other DNA
  misc_feature 17..23: note = n stands for any base
  misc_feature 27..29: note = n stands for any base
  misc_feature 33..36: note = n stands for any base

SEQ ID NO: 61 - DNA, 68 bp, synthetic construct; identical to SEQ ID NO: 33
  source 1..68: mol_type = other DNA
  misc_feature 17..23: note = n stands for any base
  misc_feature 27..29: note = n stands for any base
  misc_feature 33..36: note = n stands for any base

SEQ ID NO: 62 - DNA, 68 bp, synthetic construct; identical to SEQ ID NO: 34
  source 1..68: mol_type = other DNA
  misc_feature 17..23: note = n stands for any base
  misc_feature 27..29: note = n stands for any base
  misc_feature 33..36: note = n stands for any base

SEQ ID NO: 63 - DNA, 68 bp, synthetic construct; identical to SEQ ID NO: 35
  source 1..68: mol_type = other DNA
  misc_feature 17..23: note = n stands for any base
  misc_feature 27..29: note = n stands for any base
  misc_feature 33..36: note = n stands for any base

SEQ ID NO: 64 - DNA, 66 bp, synthetic construct; identical to SEQ ID NO: 36
  source 1..66: mol_type = other DNA
  misc_feature 17..23: note = n stands for any base
  misc_feature 27..29: note = n stands for any base
  misc_feature 33..36: note = n stands for any base

SEQ ID NO: 65 - DNA, 68 bp, synthetic construct; identical to SEQ ID NO: 37
  source 1..68: mol_type = other DNA
  misc_feature 17..23: note = n stands for any base
  misc_feature 27..29: note = n stands for any base
  misc_feature 33..36: note = n stands for any base

SEQ ID NO: 66 - DNA, 68 bp, synthetic construct
  source 1..68: mol_type = other DNA
  misc_feature 17..23: note = n stands for any base
  misc_feature 27..29: note = n stands for any base
  misc_feature 33..36: note = n stands for any base
gacgctcttccgatctnnnnnnnwwsnnnwwwnnnnsaccgtttcacgcgtaagtttaggacacctca

SEQ ID NO: 67 - DNA, 68 bp, synthetic construct
  source 1..68: mol_type = other DNA
  misc_feature 17..23: note = n stands for any base
  misc_feature 27..29: note = n stands for any base
  misc_feature 33..36: note = n stands for any base
gacgctcttccgatctnnnnnnnwwsnnnwwwnnnnsacaaggccacgcgtaagtttaggacacctca

SEQ ID NO: 68 - DNA, 68 bp, synthetic construct
  source 1..68: mol_type = other DNA
  misc_feature 17..23: note = n stands for any base
  misc_feature 27..29: note = n stands for any base
  misc_feature 33..36: note = n stands for any base
gacgctcttccgatctnnnnnnnwwsnnnwwwnnnnsactccgaaacgcgtaagtttaggacacctca

SEQ ID NO: 69 - DNA, 66 bp, synthetic construct; identical to SEQ ID NO: 20
  source 1..66: mol_type = other DNA
  misc_feature 17..23: note = n stands for any base
  misc_feature 27..29: note = n stands for any base
  misc_feature 33..36: note = n stands for any base

SEQ ID NO: 70 - DNA, 66 bp, synthetic construct; identical to SEQ ID NO: 21
  source 1..66: mol_type = other DNA
  misc_feature 17..23: note = n stands for any base
  misc_feature 27..29: note = n stands for any base
  misc_feature 33..36: note = n stands for any base

SEQ ID NO: 71 - DNA, 66 bp, synthetic construct; identical to SEQ ID NO: 22
  source 1..66: mol_type = other DNA
  misc_feature 17..23: note = n stands for any base
  misc_feature 27..29: note = n stands for any base
  misc_feature 33..36: note = n stands for any base

SEQ ID NO: 72 - DNA, 66 bp, synthetic construct; identical to SEQ ID NO: 23
  source 1..66: mol_type = other DNA
  misc_feature 17..23: note = n stands for any base
  misc_feature 27..29: note = n stands for any base
  misc_feature 33..36: note = n stands for any base

SEQ ID NO: 73 - DNA, 66 bp, synthetic construct; identical to SEQ ID NO: 26
  source 1..66: mol_type = other DNA
  misc_feature 17..23: note = n stands for any base
  misc_feature 27..29: note = n stands for any base
  misc_feature 33..36: note = n stands for any base

SEQ ID NO: 74 - DNA, 66 bp, synthetic construct; identical to SEQ ID NO: 24
  source 1..66: mol_type = other DNA
  misc_feature 17..23: note = n stands for any base
  misc_feature 27..29: note = n stands for any base
  misc_feature 33..36: note = n stands for any base

SEQ ID NO: 75 - DNA, 66 bp, synthetic construct; identical to SEQ ID NO: 41
  source 1..66: mol_type = other DNA
  misc_feature 17..23: note = n stands for any base
  misc_feature 27..29: note = n stands for any base
  misc_feature 33..36: note = n stands for any base

SEQ ID NO: 76 - DNA, 66 bp, synthetic construct; identical to SEQ ID NO: 38
  source 1..66: mol_type = other DNA
  misc_feature 17..23: note = n stands for any base
  misc_feature 27..29: note = n stands for any base
  misc_feature 33..36: note = n stands for any base

SEQ ID NO: 77 - DNA, 66 bp, synthetic construct; identical to SEQ ID NO: 40
  source 1..66: mol_type = other DNA
  misc_feature 17..23: note = n stands for any base
  misc_feature 27..29: note = n stands for any base
  misc_feature 33..36: note = n stands for any base

SEQ ID NO: 78 - DNA, 66 bp, synthetic construct; identical to SEQ ID NO: 42
  source 1..66: mol_type = other DNA
  misc_feature 17..23: note = n stands for any base
  misc_feature 27..29: note = n stands for any base
  misc_feature 33..36: note = n stands for any base

SEQ ID NO: 79 - DNA, 66 bp, synthetic construct; identical to SEQ ID NO: 43
  source 1..66: mol_type = other DNA
  misc_feature 17..23: note = n stands for any base
  misc_feature 27..29: note = n stands for any base
  misc_feature 33..36: note = n stands for any base

SEQ ID NO: 80 - DNA, 66 bp, synthetic construct; identical to SEQ ID NO: 44
  source 1..66: mol_type = other DNA
  misc_feature 17..23: note = n stands for any base
  misc_feature 27..29: note = n stands for any base
  misc_feature 33..36: note = n stands for any base

SEQ ID NO: 81 - DNA, 66 bp, synthetic construct; identical to SEQ ID NO: 45
  source 1..66: mol_type = other DNA
  misc_feature 17..23: note = n stands for any base
  misc_feature 27..29: note = n stands for any base
  misc_feature 33..36: note = n stands for any base

SEQ ID NO: 82 - DNA, 66 bp, synthetic construct; identical to SEQ ID NO: 46
  source 1..66: mol_type = other DNA
  misc_feature 17..23: note = n stands for any base
  misc_feature 27..29: note = n stands for any base
  misc_feature 33..36: note = n stands for any base

SEQ ID NO: 83 - DNA, 66 bp, synthetic construct; identical to SEQ ID NO: 47
  source 1..66: mol_type = other DNA
  misc_feature 17..23: note = n stands for any base
  misc_feature 27..29: note = n stands for any base
  misc_feature 33..36: note = n stands for any base

SEQ ID NO: 84 - DNA, 68 bp, synthetic construct; identical to SEQ ID NO: 48
  source 1..68: mol_type = other DNA
  misc_feature 17..23: note = n stands for any base
  misc_feature 27..29: note = n stands for any base
  misc_feature 33..36: note = n stands for any base

SEQ ID NO: 85 - DNA, 66 bp, synthetic construct; identical to SEQ ID NO: 39
  source 1..66: mol_type = other DNA
  misc_feature 17..23: note = n stands for any base
  misc_feature 27..29: note = n stands for any base
  misc_feature 33..36: note = n stands for any base

SEQ ID NO: 86 - DNA, 66 bp, synthetic construct
  source 1..66: mol_type = other DNA
  misc_feature 17..23: note = n stands for any base
  misc_feature 27..29: note = n stands for any base
  misc_feature 33..36: note = n stands for any base
tgtgctcttccgatctnnnnnnnwwsnnnwwwnnnnsacgctgtagcgatatgttgagaccactcc

SEQ ID NO: 87 - DNA, 66 bp, synthetic construct
  source 1..66: mol_type = other DNA
  misc_feature 17..23: note = n stands for any base
  misc_feature 27..29: note = n stands for any base
  misc_feature 33..36: note = n stands for any base
tgtgctcttccgatctnnnnnnnwwsnnnwwwnnnnsacattatagcgatatgttgagaccactcc

SEQ ID NO: 88 - DNA, 66 bp, synthetic construct
  source 1..66: mol_type = other DNA
  misc_feature 17..23: note = n stands for any base
  misc_feature 27..29: note = n stands for any base
  misc_feature 33..36: note = n stands for any base
tgtgctcttccgatctnnnnnnnwwsnnnwwwnnnnsacgaatgagcgatatgttgagaccactcc